European Patent Specification EP 3 448 890 B1, published July 19, 2023. Title: BISPECIFIC ANTIBODIES TARGETING EGFR AND HER2. Applicant: BIOMUNEX pharmaceuticals et al. The sequence listing filed with the application follows.

SEQUENCE LISTING (38 sequences)

SEQ ID NO: 1 - protein, 120 aa, Homo sapiens [sequence omitted]

SEQ ID NO: 2 - protein, 98 aa, Homo sapiens
ASTKGPSVFPLAPSSKSTSGGTAALGCLVKDYFPEPVTVSWNSGALTSGVHTFPAVLQSSGLYSLSSVVTVPSSSLGTQTYICNVNHKPSNTKVDKKV

SEQ ID NO: 3 - protein, 34 aa, Artificial Sequence
  linker sequence
EPKSCDKTHTCPPCPAPELLGGPSTPPTPSPSGG

SEQ ID NO: 4 - protein, 119 aa, Homo sapiens
QVQLKQSGPGLVQPSQSLSITCTVSGFSLTNYGVHWVRQSPGKGLEWLGVIWSGGNTDYNTPFTSRLSINKDNSKSQVFFKMNSLQSNDTAIYYCARALTYYDYEFAYWGQGTLVTVSA

SEQ ID NO: 5 - protein, 98 aa, Homo sapiens
ASTKGPSVFPLAPSSKSTSGGTAALGCLVKDYFPEPVTVSWNSGALTSGVHTFPAVLQSSGLYSLSSVVEVPSSSLGTQTYICNVNHKPSNTKVDKKV

SEQ ID NO: 6 - protein, 15 aa, Homo sapiens
EPKSCDKTHTCPPCP

SEQ ID NO: 7 - protein, 110 aa, Homo sapiens
APELLGGPSVFLFPPKPKDTLMISRTPEVTCVVVDVSHEDPEVKFNWYVDGVEVHNAKTKPREEQYNSTYRVVSVLTVLHQDWLNGKEYKCKVSNKALPAPIEKTISKAK

SEQ ID NO: 8 - protein, 107 aa, Homo sapiens
GQPREPQVYTLPPSREEMTKNQVSLTCLVKGFYPSDIAVEWESNGQPENNYKTTPPVLDSDGSFFLYSKLTVDKSRWQQGNVFSCSVMHEALHNHYTQKSLSLSPGK

SEQ ID NO: 9 - protein, 701 aa, Artificial Sequence
  BiXAb 3486 heavy chain
EVQLVESGGGLVQPGGSLRLSCAASGFNIKDTYIHWVRQAPGKGLEWVARIYPTNGYTRYADSVKGRFTISADTSKNTAYLQMNSLRAEDTAVYYCSRWGGDGFYAMDYWGQGTLVTVSSASTKGPSVFPLAPSSKSTSGGTAALGCLVKDYFPEPVTVSWNSGALTSGVHTFPAVLQSSGLYSLSSVVTVPSSSLGTQTYICNVNHKPSNTKVDKKVEPKSCDKTHTCPPCPAPELLGGPSTPPTPSPSGGQVQLKQSGPGLVQPSQSLSITCTVSGFSLTNYGVHWVRQSPGKGLEWLGVIWSGGNTDYNTPFTSRLSINKDNSKSQVFFKMNSLQSNDTAIYYCARALTYYDYEFAYWGQGTLVTVSAASTKGPSVFPLAPSSKSTSGGTAALGCLVKDYFPEPVTVSWNSGALTSGVHTFPAVLQSSGLYSLSSVVEVPSSSLGTQTYICNVNHKPSNTKVDKKVEPKSCDKTHTCPPCPAPELLGGPSVFLFPPKPKDTLMISRTPEVTCVVVDVSHEDPEVKFNWYVDGVEVHNAKTKPREEQYNSTYRVVSVLTVLHQDWLNGKEYKCKVSNKALPAPIEKTISKAKGQPREPQVYTLPPSREEMTKNQVSLTCLVKGFYPSDIAVEWESNGQPENNYKTTPPVLDSDGSFFLYSKLTVDKSRWQQGNVFSCSVMHEALHNHYTQKSLSLSPGK

SEQ ID NO: 10 - protein, 107 aa, Homo sapiens [sequence omitted]

SEQ ID NO: 11 - protein, 107 aa, Homo sapiens [sequence omitted]

SEQ ID NO: 12 - protein, 214 aa, Homo sapiens
DIQMTQSPSSLSASVGDRVTITCRASQDVNTAVAWYQQKPGKAPKLLIYSASFLYSGVPSRFSGSRSGTDFTLTISSLQPEDFATYYCQQHYTTPPTFGQGTKVEIKRTVAAPSVFIFPPSDEQLKSGTASVVCLLNNFYPREAKVQWKVDNALQSGNSQESVTEQDSKDSTYSLSSTLTLSKADYEKHKVYACEVTHQGLSSPVTKSFNRGEC

SEQ ID NO: 13 - protein, 107 aa, Homo sapiens
DILLTQSPVILSVSPGERVSFSCRASQSIGTNIHWYQQRTNGSPRLLIKYASESISGIPSRFSGSGSGTDFTLSINSVESEDIADYYCQQNNNWPTTFGAGTKLELK

SEQ ID NO: 14 - protein, 107 aa, Homo sapiens
RTVAAPAVFIFPPSDEQLKSGTASVVCLLKNFYPREAKVQWKVDNALQSGNSQESVTEQDSKDSTYSLSSTLTLSKADYEKHKVYACEVTHQGLSSPVTKSFNRGEC

SEQ ID NO: 15 - protein, 214 aa, Homo sapiens
DILLTQSPVILSVSPGERVSFSCRASQSIGTNIHWYQQRTNGSPRLLIKYASESISGIPSRFSGSGSGTDFTLSINSVESEDIADYYCQQNNNWPTTFGAGTKLELKRTVAAPAVFIFPPSDEQLKSGTASVVCLLKNFYPREAKVQWKVDNALQSGNSQESVTEQDSKDSTYSLSSTLTLSKADYEKHKVYACEVTHQGLSSPVTKSFNRGEC

SEQ ID NO: 16 - protein, 34 aa, Artificial Sequence
  linker sequence
EPKSCDKTHTSPPSPAPELLGGPSTPPTPSPSGG

SEQ ID NO: 17 - protein, 701 aa, Artificial Sequence
  BiXAb 3489 heavy chain
EVQLVESGGGLVQPGGSLRLSCAASGFNIKDTYIHWVRQAPGKGLEWVARIYPTNGYTRYADSVKGRFTISADTSKNTAYLQMNSLRAEDTAVYYCSRWGGDGFYAMDYWGQGTLVTVSSASTKGPSVFPLAPSSKSTSGGTAALGCLVKDYFPEPVTVSWNSGALTSGVHTFPAVLQSSGLYSLSSVVTVPSSSLGTQTYICNVNHKPSNTKVDKKVEPKSCDKTHTSPPSPAPELLGGPSTPPTPSPSGGQVQLKQSGPGLVQPSQSLSITCTVSGFSLTNYGVHWVRQSPGKGLEWLGVIWSGGNTDYNTPFTSRLSINKDNSKSQVFFKMNSLQSNDTAIYYCARALTYYDYEFAYWGQGTLVTVSAASTKGPSVFPLAPSSKSTSGGTAALGCLVKDYFPEPVTVSWNSGALTSGVHTFPAVLQSSGLYSLSSVVEVPSSSLGTQTYICNVNHKPSNTKVDKKVEPKSCDKTHTCPPCPAPELLGGPSVFLFPPKPKDTLMISRTPEVTCVVVDVSHEDPEVKFNWYVDGVEVHNAKTKPREEQYNSTYRVVSVLTVLHQDWLNGKEYKCKVSNKALPAPIEKTISKAKGQPREPQVYTLPPSREEMTKNQVSLTCLVKGFYPSDIAVEWESNGQPENNYKTTPPVLDSDGSFFLYSKLTVDKSRWQQGNVFSCSVMHEALHNHYTQKSLSLSPGK

SEQ ID NO: 18 - protein, 701 aa, Artificial Sequence
  BiXAb 3732 heavy chain
QVQLKQSGPGLVQPSQSLSITCTVSGFSLTNYGVHWVRQSPGKGLEWLGVIWSGGNTDYNTPFTSRLSINKDNSKSQVFFKMNSLQSNDTAIYYCARALTYYDYEFAYWGQGTLVTVSAASTKGPSVFPLAPSSKSTSGGTAALGCLVKDYFPEPVTVSWNSGALTSGVHTFPAVLQSSGLYSLSSVVEVPSSSLGTQTYICNVNHKPSNTKVDKKVEPKSCDKTHTCPPCPAPELLGGPSTPPTPSPSGGEVQLVESGGGLVQPGGSLRLSCAASGFNIKDTYIHWVRQAPGKGLEWVARIYPTNGYTRYADSVKGRFTISADTSKNTAYLQMNSLRAEDTAVYYCSRWGGDGFYAMDYWGQGTLVTVSSASTKGPSVFPLAPSSKSTSGGTAALGCLVKDYFPEPVTVSWNSGALTSGVHTFPAVLQSSGLYSLSSVVTVPSSSLGTQTYICNVNHKPSNTKVDKKVEPKSCDKTHTCPPCPAPELLGGPSVFLFPPKPKDTLMISRTPEVTCVVVDVSHEDPEVKFNWYVDGVEVHNAKTKPREEQYNSTYRVVSVLTVLHQDWLNGKEYKCKVSNKALPAPIEKTISKAKGQPREPQVYTLPPSREEMTKNQVSLTCLVKGFYPSDIAVEWESNGQPENNYKTTPPVLDSDGSFFLYSKLTVDKSRWQQGNVFSCSVMHEALHNHYTQKSLSLSPGK

SEQ ID NO: 19 - protein, 701 aa, Artificial Sequence
  BiXAb 3732SS heavy chain
QVQLKQSGPGLVQPSQSLSITCTVSGFSLTNYGVHWVRQSPGKGLEWLGVIWSGGNTDYNTPFTSRLSINKDNSKSQVFFKMNSLQSNDTAIYYCARALTYYDYEFAYWGQGTLVTVSAASTKGPSVFPLAPSSKSTSGGTAALGCLVKDYFPEPVTVSWNSGALTSGVHTFPAVLQSSGLYSLSSVVEVPSSSLGTQTYICNVNHKPSNTKVDKKVEPKSCDKTHTSPPSPAPELLGGPSTPPTPSPSGGEVQLVESGGGLVQPGGSLRLSCAASGFNIKDTYIHWVRQAPGKGLEWVARIYPTNGYTRYADSVKGRFTISADTSKNTAYLQMNSLRAEDTAVYYCSRWGGDGFYAMDYWGQGTLVTVSSASTKGPSVFPLAPSSKSTSGGTAALGCLVKDYFPEPVTVSWNSGALTSGVHTFPAVLQSSGLYSLSSVVTVPSSSLGTQTYICNVNHKPSNTKVDKKVEPKSCDKTHTCPPCPAPELLGGPSVFLFPPKPKDTLMISRTPEVTCVVVDVSHEDPEVKFNWYVDGVEVHNAKTKPREEQYNSTYRVVSVLTVLHQDWLNGKEYKCKVSNKALPAPIEKTISKAKGQPREPQVYTLPPSREEMTKNQVSLTCLVKGFYPSDIAVEWESNGQPENNYKTTPPVLDSDGSFFLYSKLTVDKSRWQQGNVFSCSVMHEALHNHYTQKSLSLSPGK

SEQ ID NO: 20 - protein, 98 aa, Homo sapiens
ASTKGPSVFPLAPSSKSTSGGTAALGCLVKDYFPEPVTVSWNSGALTSGVHTFPAVLQSSGLYSLSSVVDVPSSSLGTQTYICNVNHKPSNTKVDKKV

SEQ ID NO: 21 - protein, 98 aa, Homo sapiens
ASTKGPSVFPLAPSSKSTSGGTAALGCLVKDYFPEPVTVSWNSGALTSGVHTFPAVLQSSGLYSLSSVVKVPSSSLGTQTYICNVNHKPSNTKVDKKV

SEQ ID NO: 22 - protein, 98 aa, Homo sapiens
ASTKGPSVFPLAPSSKSTSGGTAALGCLVKDYFPEPVTVSWNSGALTSGVHTFPAVLQSSGLYSLSSVVRVPSSSLGTQTYICNVNHKPSNTKVDKKV

SEQ ID NO: 23 - protein, 107 aa, Homo sapiens
RTVAAPAVFIFPPSDEQLKSGTASVVCLLRNFYPREAKVQWKVDNALQSGNSQESVTEQDSKDSTYSLSSTLTLSKADYEKHKVYACEVTHQGLSSPVTKSFNRGEC

SEQ ID NO: 24 - protein, 107 aa, Homo sapiens
RTVAAPAVFIFPPSDEQLKSGTASVVCLLENFYPREAKVQWKVDNALQSGNSQESVTEQDSKDSTYSLSSTLTLSKADYEKHKVYACEVTHQGLSSPVTKSFNRGEC

SEQ ID NO: 25 - protein, 107 aa, Homo sapiens
RTVAAPAVFIFPPSDEQLKSGTASVVCLLDNFYPREAKVQWKVDNALQSGNSQESVTEQDSKDSTYSLSSTLTLSKADYEKHKVYACEVTHQGLSSPVTKSFNRGEC

SEQ ID NO: 26 - protein, 119 aa, Homo sapiens
QVQLKQSGPGLVQPSQSLSITCTVSGFSLTNYGVHWVRQSPGKGLEWLGVIWSGGNTDYNTPFTSRLSINKDNSKSQVFFKMNSLQSDDTAIYYCARALTYYDYEFAYWGQGTLVTVSA

SEQ ID NO: 27 - protein, 119 aa, Homo sapiens
QVQLKQSGPGLVQPSQSLSITCTVSGFSLTNYGVHWVRQSPGKGLEWLGVIWSGGNTDYNTPFTSRLSINKDNSKSQVFFKMNSLQSEDTAIYYCARALTYYDYEFAYWGQGTLVTVSA

SEQ ID NO: 28 - protein, 9 aa, Homo sapiens
APELLGGPS

SEQ ID NO: 29 - protein, 8 aa, Homo sapiens
TPPTPSPS

SEQ ID NO: 30 - protein, 107 aa, Homo sapiens
EIVLTQSPDFQSVTPKEKVTITCRASQSIGTNIHWYQQKPDQSPKLLIKYASESISGVPSRFSGSGSGTDFTLTINSLEAEDAATYYCQQNNNWPTTFGQGTKLEIK

SEQ ID NO: 31 - protein, 107 aa, Homo sapiens
EIVLTQSPATLSLSPGERATLSCRASQSIGTNIHWYQQKPGQAPRLLIKYASESISGIPARFSGSGSGTDFTLTISSLEPEDFAVYYCQQNNNWPTTFGQGTKLEIK

SEQ ID NO: 32 - protein, 119 aa, Homo sapiens
QVQLQESGPGLVKPSETLSLTCTVSGFSLTNYGVHWVRQPPGKGLEWLGVIWSGGNTDYNTPLTSRLTISKDNSKNQVSLKLSSVTAADTAVYYCARALTYYDYEFAYWGQGTLVTVSS

SEQ ID NO: 33 - protein, 119 aa, Homo sapiens
QVQLVESGGGVVQPGRSLRLSCAVSGFSLTNYGVHWVRQAPGKGLEWLGVIWSGGNTDYNTPVTSRFTISKDNSKNTVYLQMNSLRAEDTAVYYCARALTYYDYEFAYWGQGTLVTVSS

SEQ ID NO: 34 - protein, 34 aa, Artificial Sequence
  linker sequence
EPKSCDKTHTSPPAPAPELLGGPAAPPAPAPAGG

SEQ ID NO: 35 - protein, 701 aa, Artificial Sequence
  BiXAb E06528 heavy chain
EVQLVESGGGLVQPGGSLRLSCAASGFNIKDTYIHWVRQAPGKGLEWVARIYPTNGYTRYADSVKGRFTISADTSKNTAYLQMNSLRAEDTAVYYCSRWGGDGFYAMDYWGQGTLVTVSSASTKGPSVFPLAPSSKSTSGGTAALGCLVKDYFPEPVTVSWNSGALTSGVHTFPAVLQSSGLYSLSSVVTVPSSSLGTQTYICNVNHKPSNTKVDKKVEPKSCDKTHTSPPAPAPELLGGPAAPPAPAPAGGQVQLKQSGPGLVQPSQSLSITCTVSGFSLTNYGVHWVRQSPGKGLEWLGVIWSGGNTDYNTPFTSRLSINKDNSKSQVFFKMNSLQSNDTAIYYCARALTYYDYEFAYWGQGTLVTVSAASTKGPSVFPLAPSSKSTSGGTAALGCLVKDYFPEPVTVSWNSGALTSGVHTFPAVLQSSGLYSLSSVVEVPSSSLGTQTYICNVNHKPSNTKVDKKVEPKSCDKTHTCPPCPAPELLGGPSVFLFPPKPKDTLMISRTPEVTCVVVDVSHEDPEVKFNWYVDGVEVHNAKTKPREEQYNSTYRVVSVLTVLHQDWLNGKEYKCKVSNKALPAPIEKTISKAKGQPREPQVYTLPPSREEMTKNQVSLTCLVKGFYPSDIAVEWESNGQPENNYKTTPPVLDSDGSFFLYSKLTVDKSRWQQGNVFSCSVMHEALHNHYTQKSLSLSPGK

SEQ ID NO: 36 - protein, 34 aa, Artificial Sequence
  linker sequence
  misc_feature (4)..(4): Xaa can be any naturally occurring amino acid
  misc_feature (8)..(8): Xaa can be any naturally occurring amino acid
  misc_feature (10)..(11): Xaa can be any naturally occurring amino acid
  misc_feature (14)..(14): Xaa can be any naturally occurring amino acid
  misc_feature (24)..(25): Xaa can be any naturally occurring amino acid
  misc_feature (28)..(28): Xaa can be any naturally occurring amino acid
  misc_feature (30)..(30): Xaa can be any naturally occurring amino acid
  misc_feature (32)..(32): Xaa can be any naturally occurring amino acid
EPKXCDKXHXXPPXPAPELLGGPXXPPXPXPXGG

SEQ ID NO: 37 - protein, 34 aa, Artificial Sequence
  linker sequence
EPKSCDKTHTSPPAPAPELLGGPGGPPGPGPGGG

SEQ ID NO: 38 - protein, 34 aa, Artificial Sequence
  linker sequence
EPKSCDKTHTSPPAPAPELLGGPAAPPGPAPGGG